European Patent Specification EP 3 374 386 B1, published May 29, 2024. Title: PROTEASE-ACTIVATED RECEPTOR-2 MODULATORS. Applicant: Oasis Pharmaceuticals, LLC. Application Not Yet Assigned. The sequence listing filed with the application follows.

SEQUENCE LISTING (80 sequences)

SEQ ID NO: 1 - protein, 14 aa, Artificial Sequence
  Synthetic Polypeptide
GHENSEKKRKQAIK

SEQ ID NO: 2 - protein, 14 aa, Artificial Sequence
  Synthetic Polypeptide
GDHNSEKKRKQAIK

SEQ ID NO: 3 - protein, 13 aa, Artificial Sequence
  Synthetic Polypeptide
DSEKKRKQAIKLI

SEQ ID NO: 4 - protein, 18 aa, Artificial Sequence
  Synthetic Polypeptide
RSSAIDENSEKKRKSAIK

SEQ ID NO: 5 - protein, 16 aa, Artificial Sequence
  Synthetic Polypeptide
AIDENSEKKFKSAIKL

SEQ ID NO: 6 - protein, 16 aa, Artificial Sequence
  Synthetic Polypeptide
AIHHDSEPKRKSAIKL

SEQ ID NO: 7 - protein, 16 aa, Artificial Sequence
  Synthetic Polypeptide
  MOD_RES (8)..(8): Pro is D-Proline
AIHHDSEPKRKSAIKL

SEQ ID NO: 8 - protein, 15 aa, Artificial Sequence
  Synthetic Polypeptide
  MOD_RES (8)..(8): Pro is D-Proline
AIHHDSEPRKSAAKL

SEQ ID NO: 9 - protein, 17 aa, Artificial Sequence
  Synthetic Polypeptide
  MOD_RES (17)..(17): Ile is D-Isoleucine
GLHHDSEPKRKSAIKLI

SEQ ID NO: 10 - protein, 16 aa, Artificial Sequence
  Synthetic Polypeptide
  MOD_RES (11)..(11): Lys is D-Lysine
  MOD_RES (16)..(16): Val is D-Valine
GLHHDSEPKRKSAIKV

SEQ ID NO: 11 - protein, 16 aa, Artificial Sequence
  Synthetic Polypeptide
  MOD_RES (11)..(11): Lys is D-Lysine
  MOD_RES (16)..(16): Leu is D-Leucine
PLHHDSEPKRKSAIKL

SEQ ID NO: 12 - protein, 18 aa, Artificial Sequence
  Synthetic Polypeptide
  MOD_RES (1)..(1): Lys is epsilon Lysine
  MOD_RES (12)..(12): Lys is D-Lysine
  MOD_RES (18)..(18): Ile is D-Isoleucine
KGLHHDSEPKRKSAIKLI

SEQ ID NO: 13 - protein, 18 aa, Artificial Sequence
  Synthetic Polypeptide
  MOD_RES (1)..(1): Lys is epsilon Lysine
  MOD_RES (12)..(12): Lys is D-Lysine
  MOD_RES (18)..(18): Val is D-Valine
KGLDENSEKKFKSAIKLV

SEQ ID NO: 14 - protein, 17 aa, Artificial Sequence
  Synthetic Polypeptide
  MOD_RES (1)..(1): Lys is epsilon Lysine
  MOD_RES (11)..(11): Lys is D-Lysine
  MOD_RES (17)..(17): Val is D-Valine
KLDENSEKKFKSAIKLV

SEQ ID NO: 15 - protein, 16 aa, Artificial Sequence
  Synthetic Polypeptide
  MOD_RES (11)..(11): Lys is D-Lysine
  MOD_RES (13)..(13): Xaa is Aib
  MOD_RES (16)..(16): Val is D-Valine
GLHHDSEPKRKSXIKV

SEQ ID NO: 16 - protein, 15 aa, Artificial Sequence
  Synthetic Polypeptide
  MOD_RES (11)..(11): Lys is D-Lysine
  MOD_RES (12)..(12): Ala is bAla
  MOD_RES (15)..(15): Val is D-Valine
GLHHDSEPKRKAIKV

SEQ ID NO: 17 - protein, 16 aa, Artificial Sequence
  Synthetic Polypeptide
  MISC_FEATURE (1)..(1): Xaa is aminohexanoic acid
  MOD_RES (11)..(11): Lys is D-Lysine
  MOD_RES (16)..(16): Val is D-Valine
XLHHDSEPKRKSAIKV

SEQ ID NO: 18 - protein, 17 aa, Artificial Sequence
  Synthetic Polypeptide
  MOD_RES (11)..(11): Lys is D-Lysine
  MOD_RES (13)..(13): Xaa is Aib
  MOD_RES (17)..(17): Val is D-Valine
GLHHDSEPKRKSXIKLV

SEQ ID NO: 19 - protein, 17 aa, Artificial Sequence
  Synthetic Polypeptide
  MOD_RES (1)..(1): Lys is epsilon Lysine
  MOD_RES (12)..(12): Lys is D-Lysine
KGLDENSEKKFKSAIKL

SEQ ID NO: 20 - protein, 17 aa, Artificial Sequence
  Synthetic Polypeptide
  MOD_RES (1)..(1): Lys is epsilon Lysine
KAIDENSEKKFKSAIKL

SEQ ID NO: 21 - protein, 16 aa, Artificial Sequence
  Synthetic Polypeptide
  MISC_FEATURE (1)..(1): Xaa is aminohexanoic acid
  MOD_RES (11)..(11): Lys is D-Lysine
  MOD_RES (13)..(13): Xaa is Aib
  MOD_RES (16)..(16): Val is D-Valine
XLHHDSEPKRKSXIKV

SEQ ID NO: 22 - protein, 17 aa, Artificial Sequence
  Synthetic Polypeptide
  MOD_RES (17)..(17): Val is D-Valine
GLHHDSEPKRKSAIKLV

SEQ ID NO: 23 - protein, 17 aa, Artificial Sequence
  Synthetic Polypeptide
  MOD_RES (1)..(1): Lys is epsilon Lysine
  MOD_RES (17)..(17): Val is D-Valine
KLHHDSEPKRKSAIKLV

SEQ ID NO: 24 - protein, 16 aa, Artificial Sequence
  Synthetic Polypeptide
  MOD_RES (16)..(16): Val is D-Valine
LHHDSEPKRKSAIKLV

SEQ ID NO: 25 - protein, 16 aa, Artificial Sequence
  Synthetic Polypeptide
AMDENSEKKYKSAIKL

SEQ ID NO: 26 - protein, 16 aa, Artificial Sequence
  Synthetic Polypeptide
  MISC_FEATURE (10)..(10): Xaa is citrulline
AMDENSEKKXKSAIKL

SEQ ID NO: 27 - protein, 16 aa, Artificial Sequence
  Synthetic Polypeptide
AMDENSEPKRKSAIKL

SEQ ID NO: 28 - protein, 16 aa, Artificial Sequence
  Synthetic Polypeptide
  MOD_RES (8)..(8): Pro is hydroxyproline
AMDENSEPKRKSAIKL

SEQ ID NO: 29 - protein, 17 aa, Artificial Sequence
  Synthetic Polypeptide
GLHHDSEPKRKSAIKLI

SEQ ID NO: 30 - protein, 17 aa, Artificial Sequence
  Synthetic Polypeptide
GLDENSEPKRKSAIKLI

SEQ ID NO: 31 - protein, 14 aa, Artificial Sequence
  Synthetic Polypeptide
GDENHEKKRKQAIK

SEQ ID NO: 32 - protein, 16 aa, Artificial Sequence
  Synthetic Polypeptide
PGDENSEKPKRKQAIK

SEQ ID NO: 33 - protein, 16 aa, Artificial Sequence
  Synthetic Polypeptide
GPDENSEKKPRKQAIK

SEQ ID NO: 34 - protein, 14 aa, Artificial Sequence
  Synthetic Polypeptide
  MISC_FEATURE (9)..(9): Xaa is citrulline
GDENSEKKXKQAIK

SEQ ID NO: 35 - protein, 15 aa, Artificial Sequence
  Synthetic Polypeptide
  MOD_RES (15)..(15): Ala is D-Alanine
GDENSEKKRKSAIKA

SEQ ID NO: 36 - protein, 15 aa, Artificial Sequence
  Synthetic Polypeptide
GDENSEKKRKQAIKL

SEQ ID NO: 37 - protein, 16 aa, Artificial Sequence
  Synthetic Polypeptide
GDENSEKKRKQAIKLI

SEQ ID NO: 38 - protein, 14 aa, Artificial Sequence
  Synthetic Polypeptide
GDENSEKKRKQAIK

SEQ ID NO: 39 - protein, 14 aa, Artificial Sequence
  Synthetic Polypeptide
GDENSEKRWLWAIK

SEQ ID NO: 40 - protein, 14 aa, Artificial Sequence
  Synthetic Polypeptide
GDENSEKKRKWAIK

SEQ ID NO: 41 - protein, 14 aa, Artificial Sequence
  Synthetic Polypeptide
MDENSEKKRKRAIK

SEQ ID NO: 42 - protein, 17 aa, Artificial Sequence
  Synthetic Polypeptide
  MISC_FEATURE (1)..(1): Xaa is absent, A, G, P, or an N-terminal linker
  MISC_FEATURE (2)..(2): Xaa is M, G, P, I, L, V, Nle, methionine sulfoxide (M(SO)), or methionine sulfone (M(SO2)), or absent when X1 is absent
  MISC_FEATURE (3)..(3): Xaa is D, E, H, or absent when X1 to X2 are absent
  MISC_FEATURE (4)..(4): Xaa is D, E, H, or absent when X1 to X3 are absent
  MISC_FEATURE (5)..(5): Xaa is N, D, or E
  MISC_FEATURE (6)..(7): Xaa can be any naturally occurring amino acid
  MISC_FEATURE (8)..(8): Xaa is any naturally occurring amino acid, D-amino acid thereof, Aib, hydroxyproline (Hyp), P, a proline homolog, G, or rigidifier/helix breaker moiety
  MISC_FEATURE (9)..(9): Xaa is K, R, P or absent
  MISC_FEATURE (10)..(10): Xaa is any naturally occurring amino acid or citrulline
  MISC_FEATURE (11)..(11): Xaa is K or any amino acid that makes the peptide bond between X10 and X11 uncleavable, or any amino acid that reduces positive charge
  MISC_FEATURE (12)..(12): Xaa is any naturally occurring amino acid or or bAla
  MISC_FEATURE (13)..(13): Xaa is A, S, T, G, Q, bAla, Aib, or absent
  MISC_FEATURE (14)..(14): Xaa is I, A, L, or V
  MISC_FEATURE (15)..(15): Xaa is K, I, or F
  MISC_FEATURE (16)..(16): Xaa is a hydrophobic amino acid, a D-amino acid thereof, or absent
  MISC_FEATURE (17)..(17): Xaa is a hydrophobic amino acid, a D-amino acid thereof, any amino acid that makes the peptide bond between X16 and X17 uncleavable by a protease, or absent
XXXXXXXXXXXXXXXXX

SEQ ID NO: 43 - protein, 16 aa, Artificial Sequence
  Synthetic Polypeptide
  MISC_FEATURE (1)..(1): Xaa is absent, A, G, P, or an N-terminal linker
  MISC_FEATURE (2)..(2): Xaa is M, G, P, I, L, V, Nle, methionine sulfoxide (M(SO)), or methionine sulfone (M(SO2)), or absent when X1 is absent
  MISC_FEATURE (3)..(3): Xaa is D, E, H, or absent when X1 to X2 are absent
  MISC_FEATURE (4)..(4): Xaa is D, E, H, or absent when X1 to X3 are absent
  MISC_FEATURE (5)..(5): Xaa is N, D, or E
  MISC_FEATURE (8)..(8): Xaa is any naturally occurring amino acid, or D-amino acid thereof, Aib, hydroxyproline (Hyp), P, a proline homolog, G, or rigidifier/helix breaker moiety
  MISC_FEATURE (9)..(9): Xaa is K, R, P or absent
  MISC_FEATURE (10)..(10): Xaa is any naturally occurring amino acid or citrulline
  MISC_FEATURE (11)..(11): Xaa is K or any amino acid that makes the peptide bond between X10 and X11 uncleavable, or any amino acid that reduces positive charge
  MISC_FEATURE (12)..(12): Xaa is any naturally occurring amino acid or bAla
  MISC_FEATURE (13)..(13): Xaa is A, S, T, G, Q, bAla, Aib, or absent
  MISC_FEATURE (14)..(14): Xaa is I, A, L, or V
  MISC_FEATURE (16)..(16): Xaa is a hydrophobic amino acid, a D-amino acid thereof, or absent
XXXXXSEXXXXXXXKX

SEQ ID NO: 44 - protein, 16 aa, Artificial Sequence
  Synthetic Polypeptide
  MISC_FEATURE (3)..(3): Xaa is H, D, E, or absent when X1 to X2 are absent
  MISC_FEATURE (4)..(4): Xaa is H, D, E, or absent when X1 to X3 are absent
  MISC_FEATURE (5)..(5): Xaa is D, E, or N
  MISC_FEATURE (8)..(8): Xaa is any naturally occurring amino acid or D-amino acid thereof, Aib, hydroxyproline (Hyp), P, a proline homolog, G, or rigidifier/helix breaker moiety
  MISC_FEATURE (10)..(10): Xaa is any naturally occurring amino acid or citrulline
  MISC_FEATURE (11)..(11): Xaa is K or any amino acid that makes the peptide bond between X10 and X11 uncleavable, or any amino acid that reduces positive charge
  MISC_FEATURE (12)..(12): Xaa is any naturally occurring amino acid or bAla
  MISC_FEATURE (13)..(13): Xaa is A, S, T, G, Q, N, bAla, Aib, or absent
  MISC_FEATURE (14)..(14): Xaa is I, A, L, or V
  MISC_FEATURE (15)..(15): Xaa is K, I, or F
  MISC_FEATURE (16)..(16): Xaa is a hydrophobic amino acid, a D-amino acid thereof, or any amino acid that makes the peptide bond between X15 and X16 uncleavable by a protease, or absent
AIXXXSEXKXXXXXXX

SEQ ID NO: 45 - protein, 16 aa, Artificial Sequence
  Synthetic Polypeptide
  MISC_FEATURE (3)..(3): Xaa is H, D, E, or absent when X1 to X2 are absent
  MISC_FEATURE (4)..(4): Xaa is H, D, E, or absent when X1 to X3 are absent
  MISC_FEATURE (5)..(5): Xaa is D, E, or N
  MISC_FEATURE (8)..(8): Xaa is any naturally occurring amino acid or D-amino acid thereof, Aib, hydroxyproline (Hyp), P, a proline homolog, G, or rigidifier/helix breaker moiety
  MISC_FEATURE (10)..(10): Xaa is any naturally occurring amino acid or citrulline
  MISC_FEATURE (11)..(11): Xaa is K or any amino acid that makes the peptide bond between X10 and X11 uncleavable, or any amino acid that reduces positive charge
  MISC_FEATURE (12)..(12): Xaa is any naturally occurring amino acid or bAla
  MISC_FEATURE (13)..(13): Xaa is A, S, T, G, Q, N, bAla, Aib, or absent
  MISC_FEATURE (14)..(14): Xaa is I, A, L, or V
  MISC_FEATURE (15)..(15): Xaa is K, I, or F
  MISC_FEATURE (16)..(16): Xaa is a hydrophobic amino acid, a D-amino acid thereof, or any amino acid that makes the peptide bond between X15 and X16 uncleavable by a protease, or absent
AMXXXSEXKXXXXXXX

SEQ ID NO: 46 - protein, 16 aa, Artificial Sequence
  Synthetic Polypeptide
  MISC_FEATURE (3)..(3): Xaa is H, D, E, or absent when X1 to X2 are absent
  MISC_FEATURE (4)..(4): Xaa is H, D, E, or absent when X1 to X3 are absent
  MISC_FEATURE (5)..(5): Xaa is D, E, or N
  MISC_FEATURE (8)..(8): Xaa is any naturally occurring amino acid or D-amino acid thereof, Aib, hydroxyproline (Hyp), P, a proline homolog, G, or rigidifier/helix breaker moiety
  MISC_FEATURE (10)..(10): Xaa is any naturally occurring amino acid or citrulline
  MISC_FEATURE (11)..(11): Xaa is K or any amino acid that makes the peptide bond between X10 and X11 uncleavable, or any amino acid that reduces positive charge
  MISC_FEATURE (12)..(12): Xaa is any naturally occurring amino acid or bAla
  MISC_FEATURE (13)..(13): Xaa is A, S, T, G, Q, N, bAla, Aib, or absent
  MISC_FEATURE (14)..(14): Xaa is I, A, L, or V
  MISC_FEATURE (15)..(15): Xaa is K, I, or F
  MISC_FEATURE (16)..(16): Xaa is a hydrophobic amino acid, a D-amino acid thereof, or any amino acid that makes the peptide bond between X15 and X16 uncleavable by a protease, or absent
GLXXXSEXKXXXXXXX

SEQ ID NO: 47 - protein, 15 aa, Artificial Sequence
  Synthetic Polypeptide
  MISC_FEATURE (7)..(7): Xaa is any naturally occurring amino acid or D-amino acid thereof, Aib, hydroxyproline (Hyp), P, a proline homolog, G, or rigidifier/helix breaker moiety
  MISC_FEATURE (9)..(9): Xaa is any naturally occurring amino acid or citrulline
  MISC_FEATURE (10)..(10): Xaa is K or any amino acid that makes the peptide bond between X10 and X11 uncleavable, or any amino acid that reduces positive charge
  MISC_FEATURE (11)..(11): Xaa is any naturally occurring amino acid or bAla
  MISC_FEATURE (12)..(12): Xaa is A, S, T, G, Q, N, bAla, Aib, or absent
  MISC_FEATURE (13)..(13): Xaa is I, A, L, or V
  MISC_FEATURE (14)..(14): Xaa is K, I, or F
  MISC_FEATURE (15)..(15): Xaa is a hydrophobic amino acid, a D-amino acid thereof, or any amino acid that makes the peptide bond between X15 and X16 uncleavable by a protease, or absent
GDENSEXKXXXXXXX

SEQ ID NO: 48 - protein, 15 aa, Artificial Sequence
  Synthetic Polypeptide
  MISC_FEATURE (5)..(5): Xaa can be any naturally occurring amino acid
  MISC_FEATURE (7)..(7): Xaa is any naturally occurring amino acid or D-amino acid thereof, Aib, hydroxyproline (Hyp), P, a proline homolog, G, or rigidifier/helix breaker moiety
  MISC_FEATURE (9)..(9): Xaa is any naturally occurring amino acid or citrulline
  MISC_FEATURE (10)..(10): Xaa is K or any amino acid that makes the peptide bond between X10 and X11 uncleavable, or any amino acid that reduces positive charge
  MISC_FEATURE (11)..(11): Xaa is any naturally occurring amino acid or bAla
  MISC_FEATURE (12)..(12): Xaa is A, S, T, G, Q, N, bAla, Aib, or absent
  MISC_FEATURE (13)..(13): Xaa is I, A, L, or V
  MISC_FEATURE (14)..(14): Xaa is K, I, or F
  MISC_FEATURE (15)..(15): Xaa is a hydrophobic amino acid, a D-amino acid thereof, or any amino acid that makes the peptide bond between X15 and X16 uncleavable by a protease, or absent
GDENXEXKXXXXXXX

SEQ ID NO: 49 - protein, 16 aa, Artificial Sequence
  Synthetic Polypeptide
  MISC_FEATURE (6)..(6): Xaa can be any naturally occurring amino acid
  MISC_FEATURE (8)..(8): Xaa is any naturally occurring amino acid or D-amino acid thereof, Aib, hydroxyproline (Hyp), P, a proline homolog, G, or rigidifier/helix breaker moiety
  MISC_FEATURE (10)..(10): Xaa is any naturally occurring amino acid or citrulline
  MISC_FEATURE (11)..(11): Xaa is K or any amino acid that makes the peptide bond between X10 and X11 uncleavable, or any amino acid that reduces positive charge
  MISC_FEATURE (12)..(12): Xaa is any naturally occurring amino acid or bAla
  MISC_FEATURE (13)..(13): Xaa is A, S, T, G, Q, N, bAla, Aib, or absent
  MISC_FEATURE (14)..(14): Xaa is I, A, L, or V
  MISC_FEATURE (15)..(15): Xaa is K, I, or F
  MISC_FEATURE (16)..(16): Xaa is a hydrophobic amino acid, a D-amino acid thereof, or any amino acid that makes the peptide bond between X15 and X16 uncleavable by a protease, or absent
GLHHDXEXKXXXXXXX

SEQ ID NO: 50 - protein, 16 aa, Artificial Sequence
  Synthetic Polypeptide
  MISC_FEATURE (6)..(6): Xaa can be any naturally occurring amino acid
  MISC_FEATURE (8)..(8): Xaa is any naturally occurring amino acid or D-amino acid thereof, Aib, hydroxyproline (Hyp), P, a proline homolog, G, or rigidifier/helix breaker moiety
  MISC_FEATURE (10)..(10): Xaa is any naturally occurring amino acid or citrulline
  MISC_FEATURE (11)..(11): Xaa is K or any amino acid that makes the peptide bond between X10 and X11 uncleavable, or any amino acid that reduces positive charge
  MISC_FEATURE (12)..(12): Xaa is any naturally occurring amino acid or bAla
  MISC_FEATURE (13)..(13): Xaa is A, S, T, G, Q, N, bAla, Aib, or absent
  MISC_FEATURE (14)..(14): Xaa is I, A, L, or V
  MISC_FEATURE (15)..(15): Xaa is K, I, or F
  MISC_FEATURE (16)..(16): Xaa is a hydrophobic amino acid, a D-amino acid thereof, or any amino acid that makes the peptide bond between X15 and X16 uncleavable by a protease, or absent
GLDENXEXKXXXXXXX

SEQ ID NO: 51 - protein, 16 aa, Artificial Sequence
  Synthetic Polypeptide
  MISC_FEATURE (3)..(3): Xaa is H, D, E, or absent when X1 to X2 are absent
  MISC_FEATURE (4)..(4): Xaa is H, D, E, or absent when X1 to X3 are absent
  MISC_FEATURE (5)..(5): Xaa is D, E, or N
  MISC_FEATURE (6)..(6): Xaa can be any naturally occurring amino acid
  MISC_FEATURE (8)..(8): Xaa is any naturally occurring amino acid or D-amino acid thereof, Aib, hydroxyproline (Hyp), P, a proline homolog, G, or rigidifier/helix breaker moiety
  MISC_FEATURE (10)..(10): Xaa is any naturally occurring amino acid or citrulline
  MISC_FEATURE (11)..(11): Xaa is K or any amino acid that makes the peptide bond between X10 and X11 uncleavable, or any amino acid that reduces positive charge
  MISC_FEATURE (12)..(12): Xaa is any naturally occurring amino acid or bAla
  MISC_FEATURE (16)..(16): Xaa is a hydrophobic amino acid, a D-amino acid thereof, or any amino acid that makes the peptide bond between X15 and X16 uncleavable by a protease, or absent
GLXXXXEXKXXXAIKX

SEQ ID NO: 52 - protein, 16 aa, Artificial Sequence
  Synthetic Polypeptide
  MISC_FEATURE (6)..(6): Xaa can be any naturally occurring amino acid
  MISC_FEATURE (8)..(8): Xaa is any naturally occurring amino acid or D-amino acid thereof, Aib, hydroxyproline (Hyp), P, a proline homolog, G, or rigidifier/helix breaker moiety
  MISC_FEATURE (10)..(10): Xaa is any naturally occurring amino acid or citrulline
  MISC_FEATURE (11)..(11): Xaa is K or any amino acid that makes the peptide bond between X10 and X11 uncleavable, or any amino acid that reduces positive charge
  MISC_FEATURE (12)..(12): Xaa is any naturally occurring amino acid or bAla
  MISC_FEATURE (16)..(16): Xaa is a hydrophobic amino acid, a D-amino acid thereof, or any amino acid that makes the peptide bond between X15 and X16 uncleavable by a protease, or absent
GLHHDXEXKXXXAIKX

SEQ ID NO: 53 - protein, 16 aa, Artificial Sequence
  Synthetic Polypeptide
  MISC_FEATURE (6)..(6): Xaa can be any naturally occurring amino acid
  MISC_FEATURE (8)..(8): Xaa is any naturally occurring amino acid or D-amino acid thereof, Aib, hydroxyproline (Hyp), P, a proline homolog, G, or rigidifier/helix breaker moiety
  MISC_FEATURE (10)..(10): Xaa is any naturally occurring amino acid or citrulline
  MISC_FEATURE (11)..(11): Xaa is K or any amino acid that makes the peptide bond between X10 and X11 uncleavable, or any amino acid that reduces positive charge
  MISC_FEATURE (12)..(12): Xaa is any naturally occurring amino acid or bAla
  MISC_FEATURE (16)..(16): Xaa is a hydrophobic amino acid, a D-amino acid thereof, or any amino acid that makes the peptide bond between X15 and X16 uncleavable by a protease, or absent
GLDENXEXKXXXAIKX

SEQ ID NO: 54 - protein, 16 aa, Artificial Sequence
  Synthetic Polypeptide
  MISC_FEATURE (8)..(8): Xaa is any naturally occurring amino acid or D-amino acid thereof, Aib, hydroxyproline (Hyp), P, a proline homolog, G, or rigidifier/helix breaker moiety
  MISC_FEATURE (10)..(10): Xaa is any naturally occurring amino acid or citrulline
  MISC_FEATURE (11)..(11): Xaa is K or any amino acid that makes the peptide bond between X10 and X11 uncleavable, or any amino acid that reduces positive charge
  MISC_FEATURE (12)..(12): Xaa is any naturally occurring amino acid or bAla
  MISC_FEATURE (13)..(13): Xaa is A, S, T, G, Q, N, bAla, Aib, or absent
  MISC_FEATURE (14)..(14): Xaa is I, A, L, or V
  MISC_FEATURE (15)..(15): Xaa is K, I, or F
  MISC_FEATURE (16)..(16): Xaa is a hydrophobic amino acid, a D-amino acid thereof, or any amino acid that makes the peptide bond between X15 and X16 uncleavable by a protease, or absent
GLHHDSEXKXXXXXXX

SEQ ID NO: 55 - protein, 16 aa, Artificial Sequence
  Synthetic Polypeptide
  MISC_FEATURE (8)..(8): Xaa is any naturally occurring amino acid or D-amino acid thereof, Aib, hydroxyproline (Hyp), P, a proline homolog, G, or rigidifier/helix breaker moiety
  MISC_FEATURE (10)..(10): Xaa is any naturally occurring amino acid or citrulline
  MISC_FEATURE (11)..(11): Xaa is K or any amino acid that makes the peptide bond between X10 and X11 uncleavable, or any amino acid that reduces positive charge
  MISC_FEATURE (12)..(12): Xaa is any naturally occurring amino acid or bAla
  MISC_FEATURE (13)..(13): Xaa is A, S, T, G, Q, N, bAla, Aib, or absent
  MISC_FEATURE (14)..(14): Xaa is I, A, L, or V
  MISC_FEATURE (15)..(15): Xaa is K, I, or F
  MISC_FEATURE (16)..(16): Xaa is a hydrophobic amino acid, a D-amino acid thereof, or any amino acid that makes the peptide bond between X15 and X16 uncleavable by a protease, or absent
GLDENSEXKXXXXXXX

SEQ ID NO: 56 - protein, 16 aa, Artificial Sequence
  Synthetic Polypeptide
  MISC_FEATURE (3)..(3): Xaa is H, D, E, or absent when X1 to X2 are absent
  MISC_FEATURE (4)..(4): Xaa is H, D, E, or absent when X1 to X3 are absent
  MISC_FEATURE (5)..(5): Xaa is D, E, or N
  MISC_FEATURE (8)..(8): Xaa is any naturally occurring amino acid or D-amino acid thereof, Aib, hydroxyproline (Hyp), P, a proline homolog, G, or rigidifier/helix breaker moiety
  MISC_FEATURE (10)..(10): Xaa is any naturally occurring amino acid or citrulline
  MISC_FEATURE (11)..(11): Xaa is K or any amino acid that makes the peptide bond between X10 and X11 uncleavable, or any amino acid that reduces positive charge
  MISC_FEATURE (12)..(12): Xaa is any naturally occurring amino acid or bAla
  MISC_FEATURE (16)..(16): Xaa is a hydrophobic amino acid, a D-amino acid thereof, or any amino acid that makes the peptide bond between X15 and X16 uncleavable by a protease, or absent
GLXXXSEXKXXXAIKX

SEQ ID NO: 57 - protein, 16 aa, Artificial Sequence
  Synthetic Polypeptide
  MISC_FEATURE (8)..(8): Xaa is any naturally occurring amino acid or D-amino acid thereof, Aib, hydroxyproline (Hyp), P, a proline homolog, G, or rigidifier/helix breaker moiety
  MISC_FEATURE (10)..(10): Xaa is any naturally occurring amino acid or citrulline
  MISC_FEATURE (11)..(11): Xaa is K or any amino acid that makes the peptide bond between X10 and X11 uncleavable, or any amino acid that reduces positive charge
  MISC_FEATURE (12)..(12): Xaa is any naturally occurring amino acid or bAla
  MISC_FEATURE (16)..(16): Xaa is a hydrophobic amino acid, a D-amino acid thereof, or any amino acid that makes the peptide bond between X15 and X16 uncleavable by a protease, or absent
GLHHDSEXKXXXAIKX

SEQ ID NO: 58 - protein, 16 aa, Artificial Sequence
  Synthetic Polypeptide
  MISC_FEATURE (8)..(8): Xaa is any naturally occurring amino acid or D-amino acid thereof, Aib, hydroxyproline (Hyp), P, a proline homolog, G, or rigidifier/helix breaker moiety
  MISC_FEATURE (10)..(10): Xaa is any naturally occurring amino acid or citrulline
  MISC_FEATURE (11)..(11): Xaa is K or any amino acid that makes the peptide bond between X10 and X11 uncleavable, or any amino acid that reduces positive charge
  MISC_FEATURE (12)..(12): Xaa is any naturally occurring amino acid or bAla
  MISC_FEATURE (16)..(16): Xaa is a hydrophobic amino acid, a D-amino acid thereof, or any amino acid that makes the peptide bond between X15 and X16 uncleavable by a protease, or absent
GLDENSEXKXXXAIKX

SEQ ID NO: 59 - protein, 16 aa, Artificial Sequence
  Synthetic Polypeptide
  MISC_FEATURE (1)..(1): Xaa is an N-terminal linker, A, G, P, or absent
  MISC_FEATURE (2)..(2): Xaa is M, G, P, I, L, V, Nle, methionine sulfoxide (M(SO)), or methionine sulfone (M(SO2)), or absent
  MISC_FEATURE (6)..(7): Xaa can be any naturally occurring amino acid
  MISC_FEATURE (8)..(8): Xaa is any naturally occurring amino acid or D-amino acid thereof, Aib, hydroxyproline (Hyp), P, a proline homolog, G, or rigidifier/helix breaker moiety
  MISC_FEATURE (9)..(9): Xaa is K, R, P, or absent
  MISC_FEATURE (10)..(10): Xaa is any naturally occurring amino acid or citrulline
  MISC_FEATURE (11)..(11): Xaa is K or any amino acid that makes the peptide bond between X10 and X11 uncleavable, or any amino acid that reduces positive charge
  MISC_FEATURE (12)..(12): Xaa is any naturally occurring amino acid or bAla
  MISC_FEATURE (16)..(16): Xaa is a hydrophobic amino acid, a D-amino acid thereof, or any amino acid that makes the peptide bond between X15 and X16 uncleavable by a protease, or absent
XXHHDXXXXXXXAIKX

SEQ ID NO: 60 - protein, 16 aa, Artificial Sequence
  Synthetic Polypeptide
  MISC_FEATURE (1)..(1): Xaa is an N-terminal linker, A, G, P, or absent
  MISC_FEATURE (2)..(2): Xaa is M, G, P, I, L, V, Nle, methionine sulfoxide (M(SO)), or methionine sulfone (M(SO2)), or absent
  MISC_FEATURE (8)..(8): Xaa is any naturally occurring amino acid or D-amino acid thereof, Aib, hydroxyproline (Hyp), P, a proline homolog, G, or rigidifier/helix breaker moiety
  MISC_FEATURE (10)..(10): Xaa is any naturally occurring amino acid or citrulline
  MISC_FEATURE (11)..(11): Xaa is K or any amino acid that makes the peptide bond between X10 and X11 uncleavable, or any amino acid that reduces positive charge
  MISC_FEATURE (12)..(12): Xaa is any naturally occurring amino acid or bAla
  MISC_FEATURE (13)..(13): Xaa is A, S, T, G, Q, N, bAla, Aib, or absent
  MISC_FEATURE (14)..(14): Xaa is I, A, L, or V
  MISC_FEATURE (15)..(15): Xaa is K, I, or F
  MISC_FEATURE (16)..(16): Xaa is a hydrophobic amino acid, a D-amino acid thereof, or any amino acid that makes the peptide bond between X15 and X16 uncleavable by a protease, or absent
XXHHDSEXKXXXXXXX

SEQ ID NO: 61 - protein, 16 aa, Artificial Sequence
  Synthetic Polypeptide
  MISC_FEATURE (1)..(1): Xaa is an N-terminal linker, A, G, P, or absent
  MISC_FEATURE (2)..(2): Xaa is M, G, P, I, L, V, Nle, methionine sulfoxide (M(SO)), or methionine sulfone (M(SO2)), or absent
  MISC_FEATURE (8)..(8): Xaa is any naturally occurring amino acid or D-amino acid thereof, Aib, hydroxyproline (Hyp), P, a proline homolog, G, or rigidifier/helix breaker moiety
  MISC_FEATURE (9)..(9): Xaa is K, R, P, or absent
  MISC_FEATURE (10)..(10): Xaa is any naturally occurring amino acid or citrulline
  MISC_FEATURE (11)..(11): Xaa is K or any amino acid that makes the peptide bond between X10 and X11 uncleavable, or any amino acid that reduces positive charge
  MISC_FEATURE (12)..(12): Xaa is any naturally occurring amino acid or bAla
  MISC_FEATURE (13)..(13): Xaa is A, S, T, G, Q, N, bAla, Aib, or absent
  MISC_FEATURE (14)..(14): Xaa is I, A, L, or V
  MISC_FEATURE (15)..(15): Xaa is K, I, or F
  MISC_FEATURE (16)..(16): Xaa is a hydrophobic amino acid, a D-amino acid thereof, or any amino acid that makes the peptide bond between X15 and X16 uncleavable by a protease, or absent
XXDENSEXXXXXXXXX

SEQ ID NO: 62 - protein, 16 aa, Artificial Sequence
  Synthetic Polypeptide
  MISC_FEATURE (1)..(1): Xaa is an N-terminal linker, A, G, P, or absent
  MISC_FEATURE (2)..(2): Xaa is M, G, P, I, L, V, Nle, methionine sulfoxide (M(SO)), or methionine sulfone (M(SO2)), or absent
  MISC_FEATURE (9)..(9): Xaa is K, R, P, or absent
  MISC_FEATURE (10)..(10): Xaa is any naturally occurring amino acid or citrulline
  MISC_FEATURE (11)..(11): Xaa is K or any amino acid that makes the peptide bond between X10 and X11 uncleavable, or any amino acid that reduces positive charge
  MISC_FEATURE (12)..(12): Xaa is any naturally occurring amino acid or bAla
  MISC_FEATURE (13)..(13): Xaa is A, S, T, G, Q, N, bAla, Aib, or absent
  MISC_FEATURE (14)..(14): Xaa is I, A, L, or V
  MISC_FEATURE (15)..(15): Xaa is K, I, or F
  MISC_FEATURE (16)..(16): Xaa is a hydrophobic amino acid, a D-amino acid thereof, or any amino acid that makes the peptide bond between X15 and X16 uncleavable by a protease, or absent
XXDENSEKXXXXXXXX

SEQ ID NO: 63 - protein, 16 aa, Artificial Sequence
  Synthetic Polypeptide
  MISC_FEATURE (1)..(1): Xaa is an N-terminal linker, A, G, P, or absent
  MISC_FEATURE (2)..(2): Xaa is M, G, P, I, L, V, Nle, methionine sulfoxide (M(SO)), or methionine sulfone (M(SO2)), or absent
  MISC_FEATURE (3)..(3): Xaa is H, D, E, or absent when X1 to X2 are absent
  MISC_FEATURE (4)..(4): Xaa is H, D, E, or absent when X1 to X3 are absent
  MISC_FEATURE (5)..(5): Xaa is D, E, or N
  MISC_FEATURE (6)..(7): Xaa is any naturally occurring amino acid
  MISC_FEATURE (8)..(8): Xaa is any naturally occurring amino acid or D-amino acid thereof, Aib, hydroxyproline (Hyp), P, a proline homolog, G, or rigidifier/helix breaker moiety
  MISC_FEATURE (9)..(9): Xaa is K, R, P, or absent
  MISC_FEATURE (10)..(10): Xaa is any naturally occurring amino acid or citrulline
  MISC_FEATURE (11)..(11): Xaa is K or any amino acid that makes the peptide bond between X10 and X11 uncleavable, or any amino acid that reduces positive charge
  MISC_FEATURE (12)..(12): Xaa is any naturally occurring amino acid or bAla
  MISC_FEATURE (16)..(16): Xaa is a hydrophobic amino acid, a D-amino acid thereof, or any amino acid that makes the peptide bond between X15 and X16 uncleavable by a protease, or absent
XXXXXXXXXXXXAIKX

SEQ ID NO: 64 - protein, 16 aa, Artificial Sequence
  Synthetic Polypeptide
  MISC_FEATURE (1)..(1): Xaa is an N-terminal linker, A, G, P, or absent
  MISC_FEATURE (2)..(2): Xaa is M, G, P, I, L, V, Nle, methionine sulfoxide (M(SO)), or methionine sulfone (M(SO2)), or absent
  MISC_FEATURE (3)..(3): Xaa is H, D, E, or absent when X1 to X2 are absent
  MISC_FEATURE (4)..(4): Xaa is H, D, E, or absent when X1 to X3 are absent
  MISC_FEATURE (5)..(5): Xaa is D, E, or N
  MISC_FEATURE (8)..(8): Xaa is any naturally occurring amino acid or D-amino acid thereof, Aib, hydroxyproline (Hyp), P, a proline homolog, G, or rigidifier/helix breaker moiety
  MISC_FEATURE (9)..(9): Xaa is K, R, P, or absent
  MISC_FEATURE (10)..(10): Xaa is any naturally occurring amino acid or citrulline
  MISC_FEATURE (11)..(11): Xaa is K or any amino acid that makes the peptide bond between X10 and X11 uncleavable, or any amino acid that reduces positive charge
  MISC_FEATURE (12)..(12): Xaa is any naturally occurring amino acid or bAla
  MISC_FEATURE (16)..(16): Xaa is a hydrophobic amino acid, a D-amino acid thereof, or any amino acid that makes the peptide bond between X15 and X16 uncleavable by a protease, or absent
XXXXXSEXXXXXAIKX

SEQ ID NO: 65 - protein, 16 aa, Artificial Sequence
  Synthetic Polypeptide
  MISC_FEATURE (1)..(1): Xaa is an N-terminal linker, A, G, P, or absent
  MISC_FEATURE (2)..(2): Xaa is M, G, P, I, L, V, Nle, methionine sulfoxide (M(SO)), or methionine sulfone (M(SO2)), or absent
  MISC_FEATURE (3)..(3): Xaa is H, D, E, or absent when X1 to X2 are absent
  MISC_FEATURE (4)..(4): Xaa is H, D, E, or absent when X1 to X3 are absent
  MISC_FEATURE (5)..(5): Xaa is D, E, or N
  MISC_FEATURE (8)..(8): Xaa is any naturally occurring amino acid or D-amino acid thereof, Aib, hydroxyproline (Hyp), P, a proline homolog, G, or rigidifier/helix breaker moiety
  MISC_FEATURE (9)..(9): Xaa is K, R, P, or absent
  MISC_FEATURE (10)..(10): Xaa is any naturally occurring amino acid or citrulline
  MISC_FEATURE (11)..(11): Xaa is K or any amino acid that makes the peptide bond between X10 and X11 uncleavable, or any amino acid that reduces positive charge
  MISC_FEATURE (12)..(12): Xaa is any naturally occurring amino acid or bAla
  MISC_FEATURE (13)..(13): Xaa is A, S, T, G, Q, N, bAla, Aib, or absent
  MISC_FEATURE (14)..(14): Xaa is I, A, L, or V
  MISC_FEATURE (15)..(15): Xaa is K, I, or F
  MISC_FEATURE (16)..(16): Xaa is a hydrophobic amino acid, a D-amino acid thereof, or any amino acid that makes the peptide bond between X15 and X16 uncleavable by a protease, or absent
XXXXXSEXXXXXXXXX

SEQ ID NO: 66 - protein, 16 aa, Artificial Sequence
  Synthetic Polypeptide
  MISC_FEATURE (1)..(1): Xaa is an N-terminal linker, A, G, P, or absent
  MISC_FEATURE (2)..(2): Xaa is M, G, P, I, L, V, Nle, methionine sulfoxide (M(SO)), or methionine sulfone (M(SO2)), or absent
  MISC_FEATURE (3)..(3): Xaa is H, D, E, or absent when X1 to X2 are absent
  MISC_FEATURE (4)..(4): Xaa is H, D, E, or absent when X1 to X3 are absent
  MISC_FEATURE (5)..(5): Xaa is D, E, or N
  MISC_FEATURE (6)..(7): Xaa is any naturally occurring amino acid
  MISC_FEATURE (12)..(12): Xaa is any naturally occurring amino acid or bAla
  MISC_FEATURE (13)..(13): Xaa is A, S, T, G, Q, N, bAla, Aib, or absent
  MISC_FEATURE (14)..(14): Xaa is I, A, L, or V
  MISC_FEATURE (15)..(15): Xaa is K, I, or F
  MISC_FEATURE (16)..(16): Xaa is a hydrophobic amino acid, a D-amino acid thereof, or any amino acid that makes the peptide bond between X15 and X16 uncleavable by a protease, or absent
XXXXXXXKKRKXXXXX

SEQ ID NO: 67 - protein, 16 aa, Artificial Sequence
  Synthetic Polypeptide
  MISC_FEATURE (1)..(1): Xaa is an N-terminal linker, A, G, P, or absent
  MISC_FEATURE (2)..(2): Xaa is M, G, P, I, L, V, Nle, methionine sulfoxide (M(SO)), or methionine sulfone (M(SO2)), or absent
  MISC_FEATURE (4)..(4): Xaa is H, D, E, or absent when X1 to X3 are absent
  MISC_FEATURE (5)..(5): Xaa is D, E, or N
  MISC_FEATURE (6)..(7): Xaa can be any naturally occurring amino acid
  MISC_FEATURE (8)..(8): Xaa is any naturally occurring amino acid or D-amino acid thereof, Aib, hydroxyproline (Hyp), P, a proline homolog, G, or rigidifier/helix breaker moiety
  MISC_FEATURE (10)..(10): Xaa is any naturally occurring amino acid or citrulline
  MISC_FEATURE (11)..(11): Xaa is K or any amino acid that makes the peptide bond between X10 and X11 uncleavable, or any amino acid that reduces positive charge
  MISC_FEATURE (12)..(12): Xaa is any naturally occurring amino acid or bAla
  MISC_FEATURE (16)..(16): Xaa is a hydrophobic amino acid, a D-amino acid thereof, or any amino acid that makes the peptide bond between X15 and X16 uncleavable by a protease, or absent
XXDXXXXXKXXXAIKX

SEQ ID NO: 68 - protein, 16 aa, Artificial Sequence
  Synthetic Polypeptide
  MISC_FEATURE (1)..(1): Xaa is an N-terminal linker, A, G, P, or absent
  MISC_FEATURE (3)..(3): Xaa is H, D, E, or absent when X1 to X2 are absent
  MISC_FEATURE (4)..(4): Xaa is H, D, E, or absent when X1 to X3 are absent
  MISC_FEATURE (5)..(5): Xaa is D, E, or N
  MISC_FEATURE (8)..(8): Xaa is any naturally occurring amino acid or D-amino acid thereof, Aib, hydroxyproline (Hyp), P, a proline homolog, G, or rigidifier/helix breaker moiety
  MISC_FEATURE (10)..(10): Xaa is any naturally occurring amino acid or citrulline
  MISC_FEATURE (11)..(11): Xaa is K or any amino acid that makes the peptide bond between X10 and X11 uncleavable, or any amino acid that reduces positive charge
  MISC_FEATURE (12)..(12): Xaa is any naturally occurring amino acid or bAla
  MISC_FEATURE (13)..(13): Xaa is A, S, T, G, Q, N, bAla, Aib, or absent
  MISC_FEATURE (16)..(16): Xaa is a hydrophobic amino acid, a D-amino acid thereof, or any amino acid that makes the peptide bond between X15 and X16 uncleavable by a protease, or absent
XLXXXSEXKXXXXIKX

SEQ ID NO: 69 - protein, 397 aa, Homo sapiens
MRSPSAAWLLGAAILLAASLSCSGTIQGTNRSSKGRSLIGKVDGTSHVTGKGVTVETVFSVDEFSASVLTGKLTTVFLPIVYTIVFVVGLPSNGMALWVFLFRTKKKHPAVIYMANLALADLLSVIWFPLKIAYHIHGNNWIYGEALCNVLIGFFYGNMYCSILFMTCLSVQRYWVIVNPMGHSRKKANIAIGISLAIWLLILLVTIPLYVVKQTIFIPALNITTCHDVLPEQLLVGDMFNYFLSLAIGVFLFPAFLTASAYVLMIRMLRSSAMDENSEKKRKRAIKLIVTVLAMYLICFTPSNLLLVVHYFLIKSQGQSHVYALYIVALCLSTLNSCIDPFVYYFVSHDFRDHAKNALLCRSVRTVKQMQVSLTSKKHSRKSSSYSSSSTTVKTSY

SEQ ID NO: 70 - protein, 18 aa, Artificial Sequence
  Synthetic Polypeptide
RSSAMDENSEKKRKSAIK

SEQ ID NO: 71 - protein, 6 aa, Artificial Sequence
  Synthetic Polypeptide
TFLLRN

SEQ ID NO: 72 - protein, 8 aa, Artificial Sequence
  Synthetic Polypeptide
PRSFLLRN

SEQ ID NO: 73 - protein, 6 aa, Artificial Sequence
  Synthetic Polypeptide
SLIGRL

SEQ ID NO: 74 - protein, 6 aa, Artificial Sequence
  Synthetic Polypeptide
AYPGKF

SEQ ID NO: 75 - protein, 6 aa, Artificial Sequence
  Synthetic Polypeptide
TFRGAP

SEQ ID NO: 76 - protein, 5 aa, Artificial Sequence
  Synthetic Polypeptide
AIHHD

SEQ ID NO: 77 - protein, 5 aa, Artificial Sequence
  Synthetic Polypeptide
AIDEN

SEQ ID NO: 78 - protein, 5 aa, Artificial Sequence
  Synthetic Polypeptide
GLHHD

SEQ ID NO: 79 - protein, 5 aa, Artificial Sequence
  Synthetic Polypeptide
GLDEN

SEQ ID NO: 80 - protein, 6 aa, Artificial Sequence
  Synthetic Polypeptide
SFLLRN